European Patent Specification EP 3 507 377 B1, published March 27, 2024. Title: ALLOSTERIC SPLIT TREHALASE BIOSENSOR. Applicant: University of Manitoba UTI Limited Partnership. Application Not yet available. The sequence listing filed with the application follows.

SEQUENCE LISTING (79 sequences)

SEQ ID NO: 1 - DNA, 20 bp, Artificial Sequence
  Forward primer for the Tn5 (aph) type II (kanamycin resistance) replacement for the entire TrA gene
tatggacagcaagcgaaccg

SEQ ID NO: 2 - DNA, 21 bp, Artificial Sequence
  Reverse primer for the Tn5 (aph) type II (kanamycin resistance) replacement for the entire TreA gene
tcagaagaactcgtcaagaag

SEQ ID NO: 3 - DNA, 53 bp, Artificial Sequence
  Forward primer HIS-TreAFatg-F
tataccatggcacaccatcaccatcaccatgaagaaacaccggtaacaccaca

SEQ ID NO: 4 - DNA, 32 bp, Artificial Sequence
  Reverse primer TreARtaa-R
tatacctaggttaaggtgtgggttgtgcctct

SEQ ID NO: 5 - DNA, 41 bp, Artificial Sequence
  Reverse primer TreA-BamHI-N-R
taattcctaggtcaggatcccggaacatatttctcgccttc

SEQ ID NO: 6 - DNA, 30 bp, Artificial Sequence
  Forward primer TreAFatg-F
tataccatggaagaaacaccggtaacacca

SEQ ID NO: 7 - DNA, 53 bp, Artificial Sequence
  Reverse primer TreA-TruncN-R
taattcctaggtcaatggtgatggtgatggtgcggaacatatttctcgccttc

SEQ ID NO: 8 - DNA, 50 bp, Artificial Sequence
  Forward primer TreA-TruncC-F
taattccatggcacaccatcaccatcaccataatttcaccctgccgaaag

SEQ ID NO: 9 - DNA, 38 bp, Artificial Sequence
  Forward primer TreA-SalI-C-F
taattccatggcagtcgacaatttcaccctgccgaaag

SEQ ID NO: 10 - DNA, 50 bp, Artificial Sequence
  Reverse primer TreA-HIS-R
tatacctaggttaatggtgatggtgatggtgaggtgtgggttgtgcctct

SEQ ID NO: 11 - DNA, 63 bp, Artificial Sequence
  Forward primer HA-TreA-N-F
tataccatggcatacccatacgatgttccagattacgctgtcgacgaagaaacaccggtaaca

SEQ ID NO: 12 - DNA, 64 bp, Artificial Sequence
  Reverse primer TreA-N-HA-R
tatacctaggtcaagcgtaatctggaacatcgtatgggtaggatcccggaacatatttctcgcc

SEQ ID NO: 13 - DNA, 63 bp, Artificial Sequence
  Forward primer HA-TreA-C-F
tataccatggcatacccatacgatgttccagattacgctgtcgacaatttcaccctgccgaaa

SEQ ID NO: 14 - protein, 55 aa, Artificial Sequence
  Protein G
TYKLILNGKTLKGETTTEAVDAATAEKVFKQYANDNGVDGEWTYDAATKTFTVTE

SEQ ID NO: 15 - protein, 60 aa, Artificial Sequence
  Protein A
TADNKFNKEQQNAFYEILHLPNLNEEQRNGFIQSLKDDPSQSANLLAEAKKLNDAQAPKA

SEQ ID NO: 16 - protein, 65 aa, Artificial Sequence
  Protein L
AMEEVTIKANLIFANGSTQTAEFKGTFEKATSEAYAYADTLKKDNGEWTVDVADKGYTLNIKFAG

SEQ ID NO: 17 - protein, 543 aa, Artificial Sequence
  N-terminally HIS-tagged TreA peptide
MAHHHHHHEETPVTPQPPDILLGPLFNDVQNAKLFPDQKTFADAVPNSDPLMILADYRMQQNQSGFDLRHFVNVNFTLPKEGEKYVPPEGQSLREHIDGLWPVLTRSTENTEKWDSLLPLPEPYVVPGGRFREVYYWDSYFTMLGLAESGHWDKVADMVANFAHEIDTYGHIPNGNRSYYLSRSQPPFFALMVELLAQHEGDAALKQYLPQMQKEYAYWMDGVENLQAGQQEKRVVKLQDGTLLNRYWDDRDTPRPESWVEDIATAKSNPNRPATEIYRDLRSAAASGWDFSSRWMDNPQQLNTLRTTSIVPVDLNSLMFKMEKILARASKAAGDNAMANQYETLANARQKGIEKYLWNDQQGWYADYDLKSHKVRNQLTAAALFPLYVNAAAKDRANKMATATKTHLLQPGGLNTTSVKSGQQWDAPNGWAPLQWVATEGLQNYGQKEVAMDISWHFLTNVQHTYDREKKLVEKYDVSTTGTGGGGGEYPLQDGFGWTNGVTLKMLDLICPKEQPCDNVPATRPTVKSATTQPSTKEAQPTP

SEQ ID NO: 18 - protein, 542 aa, Artificial Sequence
  C-terminally HIS-tagged TreA peptide
MEETPVTPQPPDILLGPLFNDVQNAKLFPDQKTFADAVPNSDPLMILADYRMQQNQSGFDLRHFVNVNFTLPKEGEKYVPPEGQSLREHIDGLWPVLTRSTENTEKWDSLLPLPEPYVVPGGRFREVYYWDSYFTMLGLAESGHWDKVADMVANFAHEIDTYGHIPNGNRSYYLSRSQPPFFALMVELLAQHEGDAALKQYLPQMQKEYAYWMDGVENLQAGQQEKRVVKLQDGTLLNRYWDDRDTPRPESWVEDIATAKSNPNRPATEIYRDLRSAAASGWDFSSRWMDNPQQLNTLRTTSIVPVDLNSLMFKMEKILARASKAAGDNAMANQYETLANARQKGIEKYLWNDQQGWYADYDLKSHKVRNQLTAAALFPLYVNAAAKDRANKMATATKTHLLQPGGLNTTSVKSGQQWDAPNGWAPLQWVATEGLQNYGQKEVAMDISWHFLTNVQHTYDREKKLVEKYDVSTTGTGGGGGEYPLQDGFGWTNGVTLKMLDLICPKEQPCDNVPATRPTVKSATTQPSTKEAQPTPHHHHHH

SEQ ID NO: 19 - protein, 549 aa, Artificial Sequence
  N- and C- terminally HIS-tagged TreA peptide
MAHHHHHHEETPVTPQPPDILLGPLFNDVQNAKLFPDQKTFADAVPNSDPLMILADYRMQQNQSGFDLRHFVNVNFTLPKEGEKYVPPEGQSLREHIDGLWPVLTRSTENTEKWDSLLPLPEPYVVPGGRFREVYYWDSYFTMLGLAESGHWDKVADMVANFAHEIDTYGHIPNGNRSYYLSRSQPPFFALMVELLAQHEGDAALKQYLPQMQKEYAYWMDGVENLQAGQQEKRVVKLQDGTLLNRYWDDRDTPRPESWVEDIATAKSNPNRPATEIYRDLRSAAASGWDFSSRWMDNPQQLNTLRTTSIVPVDLNSLMFKMEKILARASKAAGDNAMANQYETLANARQKGIEKYLWNDQQGWYADYDLKSHKVRNQLTAAALFPLYVNAAAKDRANKMATATKTHLLQPGGLNTTSVKSGQQWDAPNGWAPLQWVATEGLQNYGQKEVAMDISWHFLTNVQHTYDREKKLVEKYDVSTTGTGGGGGEYPLQDGFGWTNGVTLKMLDLICPKEQPCDNVPATRPTVKSATTQPSTKEAQPTPHHHHHH

SEQ ID NO: 20 - protein, 89 aa, Artificial Sequence
  N-terminally HIS-tagged N-terminal fragment of TreA peptide
MAHHHHHHEETPVTPQPPDILLGPLFNDVQNAKLFPDQKTFADAVPNSDPLMILADYRMQQNQSGFDLRHFVNVNFTLPKEGEKYVPGS

SEQ ID NO: 21 - protein, 86 aa, Artificial Sequence
  C-terminally HIS-tagged N-terminal fragment of TreA peptide
MEETPVTPQPPDILLGPLFNDVQNAKLFPDQKTFADAVPNSDPLMILADYRMQQNQSGFDLRHFVNVNFTLPKEGEKYVPHHHHHH

SEQ ID NO: 22 - protein, 477 aa, Artificial Sequence
  N-terminally HIS-tagged C-terminal fragment of TreA peptide
MAHHHHHHNFTLPKEGEKYVPPEGQSLREHIDGLWPVLTRSTENTEKWDSLLPLPEPYVVPGGRFREVYYWDSYFTMLGLAESGHWDKVADMVANFAHEIDTYGHIPNGNRSYYLSRSQPPFFALMVELLAQHEGDAALKQYLPQMQKEYAYWMDGVENLQAGQQEKRVVKLQDGTLLNRYWDDRDTPRPESWVEDIATAKSNPNRPATEIYRDLRSAAASGWDFSSRWMDNPQQLNTLRTTSIVPVDLNSLMFKMEKILARASKAAGDNAMANQYETLANARQKGIEKYLWNDQQGWYADYDLKSHKVRNQLTAAALFPLYVNAAAKDRANKMATATKTHLLQPGGLNTTSVKSGQQWDAPNGWAPLQWVATEGLQNYGQKEVAMDISWHFLTNVQHTYDREKKLVEKYDVSTTGTGGGGGEYPLQDGFGWTNGVTLKMLDLICPKEQPCDNVPATRPTVKSATTQPSTKEAQPTP

SEQ ID NO: 23 - protein, 478 aa, Artificial Sequence
  C-terminally HIS-tagged C-terminal fragment of TreA peptide
MAVNFTLPKEGEKYVPPEGQSLREHIDGLWPVLTRSTENTEKWDSLLPLPEPYVVPGGRFREVYYWDSYFTMLGLAESGHWDKVADMVANFAHEIDTYGHIPNGNRSYYLSRSQPPFFALMVELLAQHEGDAALKQYLPQMQKEYAYWMDGVENLQAGQQEKRVVKLQDGTLLNRYWDDRDTPRPESWVEDIATAKSNPNRPATEIYRDLRSAAASGWDFSSRWMDNPQQLNTLRTTSIVPVDLNSLMFKMEKILARASKAAGDNAMANQYETLANARQKGIEKYLWNDQQGWYADYDLKSHKVRNQLTAAALFPLYVNAAAKDRANKMATATKTHLLQPGGLNTTSVKSGQQWDAPNGWAPLQWVATEGLQNYGQKEVAMDISWHFLTNVQHTYDREKKLVEKYDVSTTGTGGGGGEYPLQDGFGWTNGVTLKMLDLICPKEQPCDNVPATRPTVKSATTQPSTKEAQPTPHHHHHH

SEQ ID NO: 24 - protein, 98 aa, Artificial Sequence
  N-terminally HA-tagged, C-terminally HIS-tagged N-terminal fragment of TreA peptide
MAYPYDVPDYAVDEETPVTPQPPDILLGPLFNDVQNAKLFPDQKTFADAVPNSDPLMILADYRMQQNQSGFDLRHFVNVNFTLPKEGEKYVPHHHHHH

SEQ ID NO: 25 - protein, 98 aa, Artificial Sequence
  N-terminally HIS-tagged, C-terminally HA-tagged N-terminal fragment of TreA peptide
MAHHHHHHEETPVTPQPPDILLGPLFNDVQNAKLFPDQKTFADAVPNSDPLMILADYRMQQNQSGFDLRHFVNVNFTLPKEGEKYVPGSYPYDVPDYA

SEQ ID NO: 26 - protein, 488 aa, Artificial Sequence
  N-terminally HA-tagged, C-terminally HIS-tagged C-terminal fragment of TreA peptide
MAYPYDVPDYAVDNFTLPKEGEKYVPPEGQSLREHIDGLWPVLTRSTENTEKWDSLLPLPEPYVVPGGRFREVYYWDSYFTMLGLAESGHWDKVADMVANFAHEIDTYGHIPNGNRSYYLSRSQPPFFALMVELLAQHEGDAALKQYLPQMQKEYAYWMDGVENLQAGQQEKRVVKLQDGTLLNRYWDDRDTPRPESWVEDIATAKSNPNRPATEIYRDLRSAAASGWDFSSRWMDNPQQLNTLRTTSIVPVDLNSLMFKMEKILARASKAAGDNAMANQYETLANARQKGIEKYLWNDQQGWYADYDLKSHKVRNQLTAAALFPLYVNAAAKDRANKMATATKTHLLQPGGLNTTSVKSGQQWDAPNGWAPLQWVATEGLQNYGQKEVAMDISWHFLTNVQHTYDREKKLVEKYDVSTTGTGGGGGEYPLQDGFGWTNGVTLKMLDLICPKEQPCDNVPATRPTVKSATTQPSTKEAQPTPHHHHHH

SEQ ID NO: 27 - protein, 488 aa, Artificial Sequence
  N-terminally HIS-tagged, C-terminally HA-tagged C-terminal fragment of TreA peptide
MAHHHHHHNFTLPKEGEKYVPPEGQSLREHIDGLWPVLTRSTENTEKWDSLLPLPEPYVVPGGRFREVYYWDSYFTMLGLAESGHWDKVADMVANFAHEIDTYGHIPNGNRSYYLSRSQPPFFALMVELLAQHEGDAALKQYLPQMQKEYAYWMDGVENLQAGQQEKRVVKLQDGTLLNRYWDDRDTPRPESWVEDIATAKSNPNRPATEIYRDLRSAAASGWDFSSRWMDNPQQLNTLRTTSIVPVDLNSLMFKMEKILARASKAAGDNAMANQYETLANARQKGIEKYLWNDQQGWYADYDLKSHKVRNQLTAAALFPLYVNAAAKDRANKMATATKTHLLQPGGLNTTSVKSGQQWDAPNGWAPLQWVATEGLQNYGQKEVAMDISWHFLTNVQHTYDREKKLVEKYDVSTTGTGGGGGEYPLQDGFGWTNGVTLKMLDLICPKEQPCDNVPATRPTVKSATTQPSTKEAQPTPGSYPYDVPDYA

SEQ ID NO: 28 - protein, 148 aa, Artificial Sequence
  N-terminally HIS-tagged N-terminal fragment of TreA with C-terminal fusion with immunoglobulin binding Domain B1 of protein G of Streptococcus
MAHHHHHHEETPVTPQPPDILLGPLFNDVQNAKLFPDQKTFADAVPNSDPLMILADYRMQQNQSGFDLRHFVNVNFTLPKEGEKYVPGSVPGSTYKLILNGKTLKGETTTEAVDAATAEKVFKQYANDNGVDGEWTYDAATKTFTVTE

SEQ ID NO: 29 - protein, 267 aa, Artificial Sequence
  N-terminally HIS-tagged N-terminal fragment of TreA with C-terminal fusion with immunoglobulin binding Domain B1 of protein G of Streptococcus
MAHHHHHHNFTLPKEGEKYVPPEGQSLREHIDGLWPVLTRSTENTEKWDSLLPLPEPYVVPGGRFREVYYWDSYFTMLGLAESGHWDKVADMVANFAHEIDTYGHIPNGNRSYYLSRSQPPFFALMVELLAQHEGDAALKQYLPQMQKEYAYWMDGVENLQAGQQEKRVVKLQDGTLLNRYWDDRDTPRPESWVEDIATAKSNPNRPATEIYRDLRSAAASGWDFSSRWMDNPQQLNTLRTTSIVPVDLNSLMFKMEKILARASKAA

SEQ ID NO: 30 - protein, 320 aa, Artificial Sequence
  HIV capside protein P24 fused N-terminally to the N-terminal fragment of TreA peptide, C-terminal HIS-tag
MEPIVQNIQGQMVHQAISPRTLNAWVKVVEEKAFSPEVIPMFSALSEGATPQDLNTMLNTVGGHQAAMQMLKETINEEAAEWDRVHPVHAGPIAPGQMREPRGSDIAGTTSTLQEQIGWMTNNPPIPVGEIYKRWIILGLNKIVRMYSPTSILDIRQGPKEPFRDYVDRFYKTLRAEQASQEVKNAMTETLLVQNANPDCKTILKALGPAATLEEMMTACQGVGGPGHKARVLVDEETPVTPQPPDILLGPLFNDVQNAKLFPDQKTFADAVPNSDPLMILADYRMQQNQSGFDLRHFVNVNFTLPKEGEKYVPHHHHHH

SEQ ID NO: 31 - protein, 710 aa, Artificial Sequence
  HIV capside protein P24 fused N-terminally to the C-terminal fragment of TreA peptide, with C-terminal HIS-tag
MEPIVQNIQGQMVHQAISPRTLNAWVKVVEEKAFSPEVIPMFSALSEGATPQDLNTMLNTVGGHQAAMQMLKETINEEAAEWDRVHPVHAGPIAPGQMREPRGSDIAGTTSTLQEQIGWMTNNPPIPVGEIYKRWIILGLNKIVRMYSPTSILDIRQGPKEPFRDYVDRFYKTLRAEQASQEVKNAMTETLLVQNANPDCKTILKALGPAATLEEMMTACQGVGGPGHKARVLVDNFTLPKEGEKYVPPEGQSLREHIDGLWPVLTRSTENTEKWDSLLPLPEPYVVPGGRFREVYYWDSYFTMLGLAESGHWDKVADMVANFAHEIDTYGHIPNGNRSYYLSRSQPPFFALMVELLAQHEGDAALKQYLPQMQKEYAYWMDGVENLQAGQQEKRVVKLQDGTLLNRYWDDRDTPRPESWVEDIATAKSNPNRPATEIYRDLRSAAASGWDFSSRWMDNPQQLNTLRTTSIVPVDLNSLMFKMEKILARASKAAGDNAMANQYETLANARQKGIEKYLWNDQQGWYADYDLKSHKVRNQLTAAALFPLYVNAAAKDRANKMATATKTHLLQPGGLNTTSVKSGQQWDAPNGWAPLQWVATEGLQNYGQKEVAMDISWHFLTNVQHTYDREKKLVEKYDVSTTGTGGGGGEYPLQDGFGWTNGVTLKMLDLICPKEQPCDNVPATRPTVKSATTQPSTKEAQPTPHHHHHH

SEQ ID NO: 32 - protein, 154 aa, Artificial Sequence
  N-terminally HIS-tagged N-terminus of TreA peptide, C-terminally fused with the immunoglobulin binding domain of protein A
MAHHHHHHEETPVTPQPPDILLGPLFNDVQNAKLFPDQKTFADAVPNSDPLMILADYRMQQNQSGFDLRHFVNVNFTLPKEGEKYVPGSAMEEVTIKANLIFANGSTQTAEFKGTFEKATSEAYAYADTLKKDNGEWTVDVADKGYTLNIKFAG

SEQ ID NO: 33 - protein, 539 aa, Artificial Sequence
  N-terminally HIS-tagged C-terminus of TreA peptide, C-terminally fused with the immunoglobulin binding domain of protein A
MAHHHHHHNFTLPKEGEKYVPPEGQSLREHIDGLWPVLTRSTENTEKWDSLLPLPEPYVVPGGRFREVYYWDSYFTMLGLAESGHWDKVADMVANFAHEIDTYGHIPNGNRSYYLSRSQPPFFALMVELLAQHEGDAALKQYLPQMQKEYAYWMDGVENLQAGQQEKRVVKLQDGTLLNRYWDDRDTPRPESWVEDIATAKSNPNRPATEIYRDLRSAAASGWDFSSRWMDNPQQLNTLRTTSIVPVDLNSLMFKMEKILARASKAAGDNAMANQYETLANARQKGVEKYLWNDQQGWYADYDLKSHKVRNQLTAAALFPLYVNAAAKDRANKMATATKTHLLQPGGLNTTSVKSGQQWDAPNGWAPLQWVATEGLQNYGQKEVAMDISWHFLTNGQHTYDREKKLVEKYDVSTTGTGGGGGEYPLQDGFGWTNGVTLKMLDLICPKEQPCDNVPATRPTVKSATTQPSTKEAQPTPGSTADNKFNKEQQNAFYEILHLPNLNEEQRNGFIQSLKDDPSQSANLLAEAKKLNDAQAPKA

SEQ ID NO: 34 - protein, 149 aa, Artificial Sequence
  N-terminally HIS-tagged N-terminus of TreA peptide, C-terminally fused with the immunoglobulin binding domain of protein L
MAHHHHHHEETPVTPQPPDILLGPLFNDVQNAKLFPDQKTFADAVPNSDPLMILADYRMQQNQSGFDLRHFVNVNFTLPKEGEKYVPGSTADNKFNKEQQNAFYEILHLPNLNEEQRNGFIQSLKDDPSQSANLLAEAKKLNDAQAPKA

SEQ ID NO: 35 - protein, 544 aa, Artificial Sequence
  N-terminally HIS-tagged C-terminus of TreA peptide, C-terminally fused with the immunoglobulin binding domain of protein L
MAHHHHHHNFTLPKEGEKYVPPEGQSLREHIDGLWPVLTRSTENTEKWDSLLPLPEPYVVPGGRFREVYYWDSYFTMLGLAESGHWDKVADMVANFAHEIDTYGHIPNGNRSYYLSRSQPPFFALMVELLAQHEGDAALKQYLPQMQKEYAYWMDGVENLQAGQQEKRVVKLQDGTLLNRYWDDRDTPRPESWVEDIATAKSNPNRPATEIYRDLRSAAASGWDFSSRWMDNPQQLNTLRTTSIVPVDLNSLMFKMEKILARASKAAGDNAMANQYETLANARQKGVEKYLWNDQQGWYADYDLKSHKVRNQLTAAALFPLYVNAAAKDRANKMATATKTHLLQPGGLNTTSVKSGQQWDAPNGWAPLQWVATEGLQNYGQKEVAMDISWHFLTNGQHTYDREKKLVEKYDVSTTGTGGGGGEYPLQDGFGWTNGVTLKMLDLICPKEQPCDNVPATRPTVKSATTQPSTKEAQPTPGSAMEEVTIKANLIFANGSTQTAEFKGTFEKATSEAYAYADTLKKDNGEWTVDVADKGYTLNIKFAG

SEQ ID NO: 36 - protein, 12 aa, Artificial Sequence
  Staphylococcus aureus binding peptide SA5-1
VPHNPGLISLQG

SEQ ID NO: 37 - protein, 12 aa, Artificial Sequence
  Mycobacterium avium subsp. paratuberculosis binding peptide Mp3
NYVIHDVPRHPA

SEQ ID NO: 38 - protein, 28 aa, Artificial Sequence
  complementary coiled-coil peptide with leucine zipper motif Ei
EIAALEKEIAALEKENAALEWEIAALEK

SEQ ID NO: 39 - protein, 28 aa, Artificial Sequence
  complementary coiled-coil peptide with leucine zipper motif Ki
KIAALKEKIAALKEKNAALKWKIAALKE

SEQ ID NO: 40 - protein, 101 aa, Artificial Sequence
  N-terminally HIS-tagged N-terminal fragment of TreA with C-terminal fusion with S. aureus binding peptide aptamer, SA5-1
MAHHHHHHEETPVTPQPPDILLGPLFNDVQNAKLFPDQKTFADAVPNSDPLMILADYRMQQNQSGFDLRHFVNVNFTLPKEGEKYVPGSVPHNPGLISLQG

SEQ ID NO: 41 - protein, 100 aa, Artificial Sequence
  N-terminally HIS-tagged N-terminal fragment of TreA with C-terminal fusion with S. aureus binding peptide aptamer, SA5-1
MVPHNPGLISLQGVDEETPVTPQPPDILLGPLFNDVQNAKLFPDQKTFADAVPNSDPLMILADYRMQQNQSGFDLRHFVNVNFTLPKEGEKYVPHHHHHH

SEQ ID NO: 42 - protein, 491 aa, Artificial Sequence
  N-terminally HIS-tagged C-terminal fragment of TreA with C-terminal fusion with S. aureus binding peptide aptamer, SA5-1
MAHHHHHHNFTLPKEGEKYVPPEGQSLREHIDGLWPVLTRSTENTEKWDSLLPLPEPYVVPGGRFREVYYWDSYFTMLGLAESGHWDKVADMVANFAHEIDTYGHIPNGNRSYYLSRSQPPFFALMVELLAQHEGDAALKQYLPQMQKEYAYWMDGVENLQAGQQEKRVVKLQDGTLLNRYWDDRDTPRPESWVEDIATAKSNPNRPATEIYRDLRSAAASGWDFSSRWMDNPQQLNTLRTTSIVPVDLNSLMFKMEKILARASKAAGDNAMANQYETLANARQKGIEKYLWNDQQGWYADYDLKSHKVRNQLTAAALFPLYVNAAAKDRANKMATATKTHLLQPGGLNTTSVKSGQQWDAPNGWAPLQWVATEGLQNYGQKEVAMDISWHFLTNVQHTYDREKKLVEKYDVSTTGTGGGGGEYPLQDGFGWTNGVTLKMLDLICPKEQPCDNVPATRPTVKSATTQPSTKEAQPTPGSVPHNPGLISLQG

SEQ ID NO: 43 - protein, 490 aa, Artificial Sequence
  C-terminally HIS-tagged C-terminal fragment of TreA with N-terminal fusion with S. aureus binding peptide aptamer, SA5-1
MVPHNPGLISLQGVDNFTLPKEGEKYVPPEGQSLREHIDGLWPVLTRSTENTEKWDSLLPLPEPYVVPGGRFREVYYWDSYFTMLGLAESGHWDKVADMVANFAHEIDTYGHIPNGNRSYYLSRSQPPFFALMVELLAQHEGDAALKQYLPQMQKEYAYWMDGVENLQAGQQEKRVVKLQDGTLLNRYWDDRDTPRPESWVEDIATAKSNPNRPATEIYRDLRSAAASGWDFSSRWMDNPQQLNTLRTTSIVPVDLNSLMFKMEKILARASKAAGDNAMANQYETLANARQKGIEKYLWNDQQGWYADYDLKSHKVRNQLTAAALFPLYVNAAAKDRANKMATATKTHLLQPGGLNTTSVKSGQQWDAPNGWAPLQWVATEGLQNYGQKEVAMDISWHFLTNVQHTYDREKKLVEKYDVSTTGTGGGGGEYPLQDGFGWTNGVTLKMLDLICPKEQPCDNVPATRPTVKSATTQPSTKEAQPTPHHHHHH

SEQ ID NO: 44 - protein, 101 aa, Artificial Sequence
  N-terminally HIS-tagged N-terminal fragment of TreA with C-terminal fusion with M. avium subsp. paratuberculosis binding peptide aptamer, Mp3
MAHHHHHHEETPVTPQPPDILLGPLFNDVQNAKLFPDQKTFADAVPNSDPLMILADYRMQQNQSGFDLRHFVNVNFTLPKEGEKYVPGSNYVIHDVPRHPA

SEQ ID NO: 45 - protein, 101 aa, Artificial Sequence
  C-terminally HIS-tagged N-terminal fragment of TreA with N-terminal fusion with M. avium subsp. paratuberculosis binding peptide aptamer, Mp3
MGNYVIHDVPRHPAVDEETPVTPQPPDILLGPLFNDVQNAKLFPDQKTFADAVPNSDPLMILADYRMQQNQSGFDLRHFVNVNFTLPKEGEKYVPHHHHHH

SEQ ID NO: 46 - protein, 491 aa, Artificial Sequence
  N-terminally HIS-tagged C-terminal fragment of TreA with C-terminal fusion with M. avium subsp. paratuberculosis binding peptide aptamer, Mp3
MAHHHHHHNFTLPKEGEKYVPPEGQSLREHIDGLWPVLTRSTENTEKWDSLLPLPEPYVVPGGRFREVYYWDSYFTMLGLAESGHWDKVADMVANFAHEIDTYGHIPNGNRSYYLSRSQPPFFALMVELLAQHEGDAALKQYLPQMQKEYAYWMDGVENLQAGQQEKRVVKLQDGTLLNRYWDDRDTPRPESWVEDIATAKSNPNRPATEIYRDLRSAAASGWDFSSRWMDNPQQLNTLRTTSIVPVDLNSLMFKMEKILARASKAAGDNAMANQYETLANARQKGIEKYLWNDQQGWYADYDLKSHKVRNQLTAAALFPLYVNAAAKDRANKMATATKTHLLQPGGLNTTSVKSGQQWDAPNGWAPLQWVATEGLQNYGQKEVAMDISWHFLTNVQHTYDREKKLVEKYDVSTTGTGGGGGEYPLQDGFGWTNGVTLKMLDLICPKEQPCDNVPATRPTVKSATTQPSTKEAQPTPGSNYVIHDVPRHPA

SEQ ID NO: 47 - protein, 491 aa, Artificial Sequence
  C-terminally HIS-tagged C-terminal fragment of TreA with N-terminal fusion with M. avium subsp. paratuberculosis binding peptide aptamer, Mp3
MGNYVIHDVPRHPAVDNFTLPKEGEKYVPPEGQSLREHIDGLWPVLTRSTENTEKWDSLLPLPEPYVVPGGRFREVYYWDSYFTMLGLAESGHWDKVADMVANFAHEIDTYGHIPNGNRSYYLSRSQPPFFALMVELLAQHEGDAALKQYLPQMQKEYAYWMDGVENLQAGQQEKRVVKLQDGTLLNRYWDDRDTPRPESWVEDIATAKSNPNRPATEIYRDLRSAAASGWDFSSRWMDNPQQLNTLRTTSIVPVDLNSLMFKMEKILARASKAAGDNAMANQYETLANARQKGIEKYLWNDQQGWYADYDLKSHKVRNQLTAAALFPLYVNAAAKDRANKMATATKTHLLQPGGLNTTSVKSGQQWDAPNGWAPLQWVATEGLQNYGQKEVAMDISWHFLTNVQHTYDREKKLVEKYDVSTTGTGGGGGEYPLQDGFGWTNGVTLKMLDLICPKEQPCDNVPATRPTVKSATTQPSTKEAQPTPHHHHHH

SEQ ID NO: 48 - protein, 817 aa, Artificial Sequence
  N-terminally HIS-tagged TreA C-terminally fused with Listeria monocytogenes ActA protein specific single chain fragment variable
MGKYLLPTAAAGLLLLAAQPAMAEVQLVESGGGVVQPGRSLRLSCAASGFAFSSYGMHWVRQAPGKGLEWVAAISYDGSNKYYADSVKGRFTISRDNSKNTLYLQMNSLRAEDTAVYYCARQADTKYFWGQGTLVTVSSGGGGSGGGGSGGSALSSELTQDPAVSVALGQTVRITCQGDSLRSYYASWYQQKPGQAPVLVIYGKNNRPSGIPDRFSGSSSGNTASLTITGAQAEDEADYYCNSRDSSGNVFGGGTKLTVLGAAAVDGGGSGGGSGGGETPVTPQPPDILLGPLFNDVQNAKLFPDQKTFADAVPNSDPLMILADYRMQQNQSGFDLRHFVNVNFTLPKEGEKYVPPEGQSLREHIDGLWPVLTRSTENTEKWDSLLPLPEPYVVPGGRFREVYYWDSYFTMLGLAESGHWDKVADMVANFAHEIDTYGHIPNGNRSYYLSRSQPPFFALMVELLAQHEGDAALKQYLPQMQKEYAYWMDGVENLQAGQQEKRVVKLQDGTLLNRYWDDRDTPRPESWVEDIATAKSNPNRPATEIYRDLRSAAASGWDFSSRWMDNPQQLNTLRTTSIVPVDLNSLMFKMEKILARASKAAGDNAMANQYETLANARQKGIEKYLWNDQQGWYADYDLKSHKVRNQLTAAALFPLYVNAAAKDRANKMATATKTHLLQPGGLNTTSVKSGQQWDAPNGWAPLQWVATEGLQNYGQKEVAMDISWHFLTNVQHTYDREKKLVEKYDVSTTGTGGGGGEYPLQDGFGWTNGVTLKMLDLICPKEQPCDNVPATRPTVKSATTQPSTKEAQPTPHHHHHH

SEQ ID NO: 49 - protein, 351 aa, Artificial Sequence
  terminally HIS-tagged N-terminal fragment of TreA C-terminally fused with Listeria monocytogenes ActA protein specific single chain fragment variable
MGKYLLPTAAAGLLLLAAQPAMAEVQLVESGGGVVQPGRSLRLSCAASGFAFSSYGMHWVRQAPGKGLEWVAAISYDGSNKYYADSVKGRFTISRDNSKNTLYLQMNSLRAEDTAVYYCARQADTKYFWGQGTLVTVSSGGGGSGGGGSGGSALSSELTQDPAVSVALGQTVRITCQGDSLRSYYASWYQQKPGQAPVLVIYGKNNRPSGIPDRFSGSSSGNTASLTITGAQAEDEADYYCNSRDSSGNVFGGGTKLTVLGAAAVDEETPVTPQPPDILLGPLFNDVQNAKLFPDQKTFADAVPNSDPLMILADYRMQQNQSGFDLRHFVNVNFTLPKEGEKYVPHHHHHH

SEQ ID NO: 50 - protein, 741 aa, Artificial Sequence
  N-terminally HIS-tagged C-terminal fragment of TreA C-terminally fused with Listeria monocytogenes ActA protein specific single chain fragment variable
MGKYLLPTAAAGLLLLAAQPAMAEVQLVESGGGVVQPGRSLRLSCAASGFAFSSYGMHWVRQAPGKGLEWVAAISYDGSNKYYADSVKGRFTISRDNSKNTLYLQMNSLRAEDTAVYYCARQADTKYFWGQGTLVTVSSGGGGSGGGGSGGSALSSELTQDPAVSVALGQTVRITCQGDSLRSYYASWYQQKPGQAPVLVIYGKNNRPSGIPDRFSGSSSGNTASLTITGAQAEDEADYYCNSRDSSGNVFGGGTKLTVLGAAAVDNFTLPKEGEKYVPPEGQSLREHIDGLWPVLTRSTENTEKWDSLLPLPEPYVVPGGRFREVYYWDSYFTMLGLAESGHWDKVADMVANFAHEIDTYGHIPNGNRSYYLSRSQPPFFALMVELLAQHEGDAALKQYLPQMQKEYAYWMDGVENLQAGQQEKRVVKLQDGTLLNRYWDDRDTPRPESWVEDIATAKSNPNRPATEIYRDLRSAAASGWDFSSRWMDNPQQLNTLRTTSIVPVDLNSLMFKMEKILARASKAAGDNAMANQYETLANARQKGIEKYLWNDQQGWYADYDLKSHKVRNQLTAAALFPLYVNAAAKDRANKMATATKTHLLQPGGLNTTSVKSGQQWDAPNGWAPLQWVATEGLQNYGQKEVAMDISWHFLTNVQHTYDREKKLVEKYDVSTTGTGGGGGEYPLQDGFGWTNGVTLKMLDLICPKEQPCDNVPATRPTVKSATTQPSTKEAQPTPHHHHHH

SEQ ID NO: 51 - protein, 220 aa, Artificial Sequence
  N-terminally HIS-tagged N-terminal fragment of TreA C-terminally fused with the ATP synthase epsilon subunit of Geobacillus
MAHHHHHHEETPVTPQPPDILLGPLFNDVQNAKLFPDQKTFADAVPNSDPLMILADYRMQQNQSGFDLRHFVNVNFTLPKEGEKYVPGSKTIHVSVVTPDGPVYEDDVEMVSVKAKSGELGILPGHIPLVAPLEISAARLKKGGKTQYIAVSGGFLEVRPDNVTILAQAAERAEDIDVLRAKARKSGRTPLQSQQDDIDFKRAELALKRAMNRLSVAEMK

SEQ ID NO: 52 - protein, 610 aa, Artificial Sequence
  N-terminally HIS-tagged C-terminal fragment of TreA C-terminally fused with the ATP synthase epsilon subunit of Geobacillus
MAHHHHHHNFTLPKEGEKYVPPEGQSLREHIDGLWPVLTRSTENTEKWDSLLPLPEPYVVPGGRFREVYYWDSYFTMLGLAESGHWDKVADMVANFAHEIDTYGHIPNGNRSYYLSRSQPPFFALMVELLAQHEGDAALKQYLPQMQKEYAYWMDGVENLQAGQQEKRVVKLQDGTLLNRYWDDRDTPRPESWVEDIATAKSNPNRPATEIYRDLRSAAASGWDFSSRWMDNPQQLNTLRTTSIVPVDLNSLMFKMEKILARASKAAGDNAMANQYETLANARQKGIEKYLWNDQQGWYADYDLKSHKVRNQLTAAALFPLYVNAAAKDRANKMATATKTHLLQPGGLNTTSVKSGQQWDAPNGWAPLQWVATEGLQNYGQKEVAMDISWHFLTNVQHTYDREKKLVEKYDVSTTGTGGGGGEYPLQDGFGWTNGVTLKMLDLICPKEQPCDNVPATRPTVKSATTQPSTKEAQPTPGSKTIHVSVVTPDGPVYEDDVEMVSVKAKSGELGILPGHIPLVAPLEISAARLKKGGKTQYIAVSGGFLEVRPDNVTILAQAAERAEDIDVLRAKARKSGRTPLQSQQDDIDFKRAELALKRAMNRLSVAEMK

SEQ ID NO: 53 - protein, 121 aa, Artificial Sequence
  N-terminally HIS-tagged N-terminal fragment of TreA with C-terminal fusion with leucine zipper 1
MAHHHHHHEETPVTPQPPDILLGPLFNDVQNAKLFPDQKTFADAVPNSDPLMILADYRMQQNQSGFDLRHFVNVNFTLPKEGEKYVPGSVPGSKIAALKEKIAALKEKNAALKWKIAALKE

SEQ ID NO: 54 - protein, 507 aa, Artificial Sequence
  N-terminally HIS-tagged N-terminal fragment of TreA with C-terminal fusion leucine zipper 2
MAHHHHHHNFTLPKEGEKYVPPEGQSLREHIDGLWPVLTRSTENTEKWDSLLPLPEPYVVPGGRFREVYYWDSYFTMLGLAESGHWDKVADMVANFAHEIDTYGHIPNGNRSYYLSRSQPPFFALMVELLAQHEGDAALKQYLPQMQKEYAYWMDGVENLQAGQQEKRVVKLQDGTLLNRYWDDRDTPRPESWVEDIATAKSNPNRPATEIYRDLRSAAASGWDFSSRWMDNPQQLNTLRTTSIVPVDLNSLMFKMEKILARASKAAGDNAMANQYETLANARQKGIEKYLWNDQQGWYADYDLKSHKVRNQLTAAALFPLYVNAAAKDRANKMATATKTHLLQPGGLNTTSVKSGQQWDAPNGWAPLQWVATEGLQNYGQKEVAMDISWHFLTNVQHTYDREKKLVEKYDVSTTGTGGGGGEYPLQDGFGWTNGVTLKMLDLICPKEQPCDNVPATRPTVKSATTQPSTKEAQPTPGSEIAALEKEIAALEKENAALEWEIAALEK

SEQ ID NO: 55 - protein, 121 aa, Artificial Sequence
  N-terminally HIS-tagged N-terminal fragment of TreA with C-terminal fusion with leucine zipper 1
MAHHHHHHEETPVTPQPPDILLGPLFNDVQNAKLFPDQKTFADAVPNSDPLMILADYRMQQNQSGFDLRHFVNVNFTLPKEGEKYVPGSVPGSEIAALEKEIAALEKENAALEWEIAALEK

SEQ ID NO: 56 - protein, 507 aa, Artificial Sequence
  N-terminally HIS-tagged N-terminal fragment of TreA with C-terminal fusion leucine zipper 2
MAHHHHHHNFTLPKEGEKYVPPEGQSLREHIDGLWPVLTRSTENTEKWDSLLPLPEPYVVPGGRFREVYYWDSYFTMLGLAESGHWDKVADMVANFAHEIDTYGHIPNGNRSYYLSRSQPPFFALMVELLAQHEGDAALKQYLPQMQKEYAYWMDGVENLQAGQQEKRVVKLQDGTLLNRYWDDRDTPRPESWVEDIATAKSNPNRPATEIYRDLRSAAASGWDFSSRWMDNPQQLNTLRTTSIVPVDLNSLMFKMEKILARASKAAGDNAMANQYETLANARQKGIEKYLWNDQQGWYADYDLKSHKVRNQLTAAALFPLYVNAAAKDRANKMATATKTHLLQPGGLNTTSVKSGQQWDAPNGWAPLQWVATEGLQNYGQKEVAMDISWHFLTNVQHTYDREKKLVEKYDVSTTGTGGGGGEYPLQDGFGWTNGVTLKMLDLICPKEQPCDNVPATRPTVKSATTQPSTKEAQPTPGSKIAALKEKIAALKEKNAALKWKIAALKE

SEQ ID NO: 57 - protein, 763 aa, Artificial Sequence
  C-terminally HIS-tagged TreA N-terminally fused with bank vole prion protein
MGKKRPKPGGWNTGGSRYPGQGSPGGNRYPPQGGGTWGQPHGGGWGQPHGGGWGQPHGGGWGQPHGGGWGQGGGTHNQWNKPSKPKTNMKHVAGAAAAGAVVGGLGGYMLGSAMSRPMIHFGNDWEDRYYRENMNRYPNQVYYRPVDQYNNQNNFVHDCVNITIKQHTVTTTTKGENFTETDVKMMERVVEQMCVTQYQKESQAYYEGRSVDGGGSGGGSGGGETPVTPQPPDILLGPLFNDVQNAKLFPDQKTFADAVPNSDPLMILADYRMQQNQSGFDLRHFVNVNFTLPKEGEKYVPPEGQSLREHIDGLWPVLTRSTENTEKWDSLLPLPEPYVVPGGRFREVYYWDSYFTMLGLAESGHWDKVADMVANFAHEIDTYGHIPNGNRSYYLSRSQPPFFALMVELLAQHEGDAALKQYLPQMQKEYAYWMDGVENLQAGQQEKRVVKLQDGTLLNRYWDDRDTPRPESWVEDIATAKSNPNRPATEIYRDLRSAAASGWDFSSRWMDNPQQLNTLRTTSIVPVDLNSLMFKMEKILARASKAAGDNAMANQYETLANARQKGIEKYLWNDQQGWYADYDLKSHKVRNQLTAAALFPLYVNAAAKDRANKMATATKTHLLQPGGLNTTSVKSGQQWDAPNGWAPLQWVATEGLQNYGQKEVAMDISWHFLTNVQHTYDREKKLVEKYDVSTTGTGGGGGEYPLQDGFGWTNGVTLKMLDLICPKEQPCDNVPATRPTVKSATTQPSTKEAQPTPHHHHHH

SEQ ID NO: 58 - protein, 308 aa, Artificial Sequence
  C-terminally HIS-tagged N-terminal fragment of TreA N-terminally fused with bank vole prion protein
MGKKRPKPGGWNTGGSRYPGQGSPGGNRYPPQGGGTWGQPHGGGWGQPHGGGWGQPHGGGWGQPHGGGWGQGGGTHNQWNKPSKPKTNMKHVAGAAAAGAVVGGLGGYMLGSAMSRPMIHFGNDWEDRYYRENMNRYPNQVYYRPVDQYNNQNNFVHDCVNITIKQHTVTTTTKGENFTETDVKMMERVVEQMCVTQYQKESQAYYEGRSVDGGGSGGGSGGGEETPVTPQPPDILLGPLFNDVQNAKLFPDQKTFADAVPNSDPLMILADYRMQQNQSGFDLRHFVNVNFTLPKEGEKYVPHHHHHH

SEQ ID NO: 59 - protein, 687 aa, Artificial Sequence
  C-terminally HIS-tagged C-terminal fragment of TreA N-terminally fused with bank vole prion protein
MGKKRPKPGGWNTGGSRYPGQGSPGGNRYPPQGGGTWGQPHGGGWGQPHGGGWGQPHGGGWGQPHGGGWGQGGGTHNQWNKPSKPKTNMKHVAGAAAAGAVVGGLGGYMLGSAMSRPMIHFGNDWEDRYYRENMNRYPNQVYYRPVDQYNNQNNFVHDCVNITIKQHTVTTTTKGENFTETDVKMMERVVEQMCVTQYQKESQAYYEGRSVDNFTLPKEGEKYVPPEGQSLREHIDGLWPVLTRSTENTEKWDSLLPLPEPYVVPGGRFREVYYWDSYFTMLGLAESGHWDKVADMVANFAHEIDTYGHIPNGNRSYYLSRSQPPFFALMVELLAQHEGDAALKQYLPQMQKEYAYWMDGVENLQAGQQEKRVVKLQDGTLLNRYWDDRDTPRPESWVEDIATAKSNPNRPATEIYRDLRSAAASGWDFSSRWMDNPQQLNTLRTTSIVPVDLNSLMFKMEKILARASKAAGDNAMANQYETLANARQKGIEKYLWNDQQGWYADYDLKSHKVRNQLTAAALFPLYVNAAAKDRANKMATATKTHLLQPGGLNTTSVKSGQQWDAPNGWAPLQWVATEGLQNYGQKEVAMDISWHFLTNVQHTYDREKKLVEKYDVSTTGTGGGGGEYPLQDGFGWTNGVTLKMLDLICPKEQPCDNVPATRPTVKSATTQPSTKEAQPTPHHHHHH

SEQ ID NO: 60 - protein, 544 aa, Artificial Sequence
  N-terminally HIS-tagged TreA with CWE scar in linker region
MAHHHHHHEETPVTPQPPDILLGPLFNDVQNAKLFPDQKTFADAVPNSDPLMILADYRMQQNQSGFDLRHFVNVNFTLPKECWEKYVPPEGQSLREHIDGLWPVLTRSTENTEKWDSLLPLPEPYVVPGGRFREVYYWDSYFTMLGLAESGHWDKVADMVANFAHEIDTYGHIPNGNRSYYLSRSQPPFFALMVELLAQHEGDAALKQYLPQMQKEYAYWMDGVENLQAGQQEKRVVKLQDGTLLNRYWDDRDTPRPESWVEDIATAKSNPNRPATEIYRDLRSAAASGWDFSSRWMDNPQQLNTLRTTSIVPVDLNSLMFKMEKILARASKAAGDNAMANQYETLANARQKGIEKYLWNDQQGWYADYDLKSHKVRNQLTAAALFPLYVNAAAKDRANKMATATKTHLLQPGGLNTTSVKSGQQWDAPNGWAPLQWVATEGLQNYGQKEVAMDISWHFLTNVQHTYDREKKLVEKYDVSTTGTGGGGGEYPLQDGFGWTNGVTLKMLDLICPKEQPCDNVPATRPTVKSATTQPSTKEAQPTP

SEQ ID NO: 61 - protein, 189 aa, Artificial Sequence
  N-terminally HIS-tagged N-terminal fragment of TreA N-terminally fused N-terminal fragment of the split intein DnaE of Nostoc punctiforme
MAHHHHHHEETPVTPQPPDILLGPLFNDVQNAKLFPDQKTFADAVPNSDPLMILADYRMQQNQSGFDLRHFVNVNFTLPKECLSYETEILTVEYGLLPIGKIVEKRIECTVYSVDNNGNIYTQPVAQWHDRGEQEVFEYCLEDGSLIRATKDHKFMTVDGQMLPIDEIFERELDLMRVDNLPNGSGGKL

SEQ ID NO: 62 - protein, 512 aa, Artificial Sequence
  C-terminally HIS-tagged C-terminal fragment of TreA N-terminally fused C-terminal fragment of the split intein DnaE of Nostoc punctiforme
MAASGGTSIKIATRKYLGKQNVYDIGVERDHNFALKNGFIASNCWEKYVPPEGQSLREHIDGLWPVLTRSTENTEKWDSLLPLPEPYVVPGGRFREVYYWDSYFTMLGLAESGHWDKVADMVANFAHEIDTYGHIPNGNRSYYLSRSQPPFFALMVELLAQHEGDAALKQYLPQMQKEYAYWMDGVENLQAGQQEKRVVKLQDGTLLNRYWDDRDTPRPESWVEDIATAKSNPNRPATEIYRDLRSAAASGWDFSSRWMDNPQQLNTLRTTSIVPVDLNSLMFKMEKILARASKAAGDNAMANQYETLANARQKGIEKYLWNDQQGWYADYDLKSHKVRNQLTAAALFPLYVNAAAKDRANKMATATKTHLLQPGGLNTTSVKSGQQWDAPNGWAPLQWVATEGLQNYGQKEVAMDISWHFLTNVQHTYDREKKLVEKYDVSTTGTGGGGGEYPLQDGFGWTNGVTLKMLDLICPKEQPCDNVPATRPTVKSATTQPSTKEAQPTPHHHHHH

SEQ ID NO: 63 - protein, 327 aa, Artificial Sequence
  C-terminally HIS-tagged N-terminal fragment of TreA N-terminally fused with human estradiol receptor fragment
MGKRSKKNSLALSLTADQMVSALLDAEPPILYSEYDPTRPFSEASMMGLLTNLADRELVHMINWAKRVPGFVDLTLHDQVHLLESAWLEILMIGLVWRSMEHPGKLLFAPNLLLDRNQGKSVEGMVEIFDMLLATSSRFRMMNLQGEEFVCLKSIILLNSGVYTFLSSTLKSLEEKDHIHRVLDKITDTLIHLMAKAGLTLQQQHQRLAQLLLILSHIRHMSNKGMEHLYSMKSKNGGSGVDEETPVTPQPPDILLGPLFNDVQNAKLFPDQKTFADAVPNSDPLMILADYRMQQNQSGFDLRHFVNVNFTLPKEGEKYVPHHHHHH

SEQ ID NO: 64 - protein, 717 aa, Artificial Sequence
  C-terminally HIS-tagged C-terminal fragment of TreA N-terminally fused with human estradiol receptor fragment
MGKRSKKNSLALSLTADQMVSALLDAEPPILYSEYDPTRPFSEASMMGLLTNLADRELVHMINWAKRVPGFVDLTLHDQVHLLESAWLEILMIGLVWRSMEHPGKLLFAPNLLLDRNQGKSVEGMVEIFDMLLATSSRFRMMNLQGEEFVCLKSIILLNSGVYTFLSSTLKSLEEKDHIHRVLDKITDTLIHLMAKAGLTLQQQHQRLAQLLLILSHIRHMSNKGMEHLYSMKSKNGGSGVDNFTLPKEGEKYVPPEGQSLREHIDGLWPVLTRSTENTEKWDSLLPLPEPYVVPGGRFREVYYWDSYFTMLGLAESGHWDKVADMVANFAHEIDTYGHIPNGNRSYYLSRSQPPFFALMVELLAQHEGDAALKQYLPQMQKEYAYWMDGVENLQAGQQEKRVVKLQDGTLLNRYWDDRDTPRPESWVEDIATAKSNPNRPATEIYRDLRSAAASGWDFSSRWMDNPQQLNTLRTTSIVPVDLNSLMFKMEKILARASKAAGDNAMANQYETLANARQKGIEKYLWNDQQGWYADYDLKSHKVRNQLTAAALFPLYVNAAAKDRANKMATATKTHLLQPGGLNTTSVKSGQQWDAPNGWAPLQWVATEGLQNYGQKEVAMDISWHFLTNVQHTYDREKKLVEKYDVSTTGTGGGGGEYPLQDGFGWTNGVTLKMLDLICPKEQPCDNVPATRPTVKSATTQPSTKEAQPTPHHHHHH

SEQ ID NO: 65 - protein, 304 aa, Artificial Sequence
  C-terminally HIS-tagged N-terminal fragment of TreA N-terminally fused with bovine interferon-gamma receptor A fragment
MASAIPGLSSVPPPTNVTIQAYNLNTVIFWDYPVILQSPMFTVQVMNYEDGKWIDACNTSDHSCNIFSVINDPSSSVWGRVKVRVGQEESVYAQSKEFILCKEGKVGPPKLGIRKKENQIIVDIFHPLITVNGKEPEAMYDDENTCYTFTYSVFVSINRSETTDKMYTKEEDCNETQCFLNIPVSSLNSQYCVSAEGVSELWAVTTEKSDELCITFSVDEETPVTPQPPDILLGPLFNDVQNAKLFPDQKTFADAVPNSDPLMILADYRMQQNQSGFDLRHFVNVNFTLPKEGEKYVPHHHHHH

SEQ ID NO: 66 - protein, 694 aa, Artificial Sequence
  C-terminally HIS-tagged C-terminal fragment of TreA N-terminally fused with bovine interferon-gamma receptor A fragment
MASAIPGLSSVPPPTNVTIQAYNLNTVIFWDYPVILQSPMFTVQVMNYEDGKWIDACNTSDHSCNIFSVINDPSSSVWGRVKVRVGQEESVYAQSKEFILCKEGKVGPPKLGIRKKENQIIVDIFHPLITVNGKEPEAMYDDENTCYTFTYSVFVSINRSETTDKMYTKEEDCNETQCFLNIPVSSLNSQYCVSAEGVSELWAVTTEKSDELCITFSVDNFTLPKEGEKYVPPEGQSLREHIDGLWPVLTRSTENTEKWDSLLPLPEPYVVPGGRFREVYYWDSYFTMLGLAESGHWDKVADMVANFAHEIDTYGHIPNGNRSYYLSRSQPPFFALMVELLAQHEGDAALKQYLPQMQKEYAYWMDGVENLQAGQQEKRVVKLQDGTLLNRYWDDRDTPRPESWVEDIATAKSNPNRPATEIYRDLRSAAASGWDFSSRWMDNPQQLNTLRTTSIVPVDLNSLMFKMEKILARASKAAGDNAMANQYETLANARQKGIEKYLWNDQQGWYADYDLKSHKVRNQLTAAALFPLYVNAAAKDRANKMATATKTHLLQPGGLNTTSVKSGQQWDAPNGWAPLQWVATEGLQNYGQKEVAMDISWHFLTNVQHTYDREKKLVEKYDVSTTGTGGGGGEYPLQDGFGWTNGVTLKMLDLICPKEQPCDNVPATRPTVKSATTQPSTKEAQPTPHHHHHH

SEQ ID NO: 67 - protein, 596 aa, Artificial Sequence
  C-terminally HIS-tagged TreA with N-terminal fusion with Amyloid beta p42 peptide
MDAEFRHDSGYEVHHQKLVFFAEDVGSNKGAIIGLMVGGVVIAVDGGGSGGGSGGGETPVTPQPPDILLGPLFNDVQNAKLFPDQKTFADAVPNSDPLMILADYRMQQNQSGFDLRHFVNVNFTLPKEGEKYVPPEGQSLREHIDGLWPVLTRSTENTEKWDSLLPLPEPYVVPGGRFREVYYWDSYFTMLGLAESGHWDKVADMVANFAHEIDTYGHIPNGNRSYYLSRSQPPFFALMVELLAQHEGDAALKQYLPQMQKEYAYWMDGVENLQAGQQEKRVVKLQDGTLLNRYWDDRDTPRPESWVEDIATAKSNPNRPATEIYRDLRSAAASGWDFSSRWMDNPQQLNTLRTTSIVPVDLNSLMFKMEKILARASKAAGDNAMANQYETLANARQKGIEKYLWNDQQGWYADYDLKSHKVRNQLTAAALFPLYVNAAAKDRANKMATATKTHLLQPGGLNTTSVKSGQQWDAPNGWAPLQWVATEGLQNYGQKEVAMDISWHFLTNVQHTYDREKKLVEKYDVSTTGTGGGGGEYPLQDGFGWTNGVTLKMLDLICPKEQPCDNVPATRPTVKSATTQPSTKEAQPTPHHHHHH

SEQ ID NO: 68 - protein, 130 aa, Artificial Sequence
  C-terminally HIS-tagged N-terminal fragment of TreA with N-terminal fusion with Amyloid beta p42 peptide
MDAEFRHDSGYEVHHQKLVFFAEDVGSNKGAIIGLMVGGVVIAVDEETPVTPQPPDILLGPLFNDVQNAKLFPDQKTFADAVPNSDPLMILADYRMQQNQSGFDLRHFVNVNFTLPKEGEKYVPHHHHHH

SEQ ID NO: 69 - protein, 520 aa, Artificial Sequence
  C-terminally HIS-tagged C-terminal fragment of TreA with N-terminal fusion with Amyloid beta p42 peptide
MDAEFRHDSGYEVHHQKLVFFAEDVGSNKGAIIGLMVGGVVIAVDNFTLPKEGEKYVPPEGQSLREHIDGLWPVLTRSTENTEKWDSLLPLPEPYVVPGGRFREVYYWDSYFTMLGLAESGHWDKVADMVANFAHEIDTYGHIPNGNRSYYLSRSQPPFFALMVELLAQHEGDAALKQYLPQMQKEYAYWMDGVENLQAGQQEKRVVKLQDGTLLNRYWDDRDTPRPESWVEDIATAKSNPNRPATEIYRDLRSAAASGWDFSSRWMDNPQQLNTLRTTSIVPVDLNSLMFKMEKILARASKAAGDNAMANQYETLANARQKGIEKYLWNDQQGWYADYDLKSHKVRNQLTAAALFPLYVNAAAKDRANKMATATKTHLLQPGGLNTTSVKSGQQWDAPNGWAPLQWVATEGLQNYGQKEVAMDISWHFLTNVQHTYDREKKLVEKYDVSTTGTGGGGGEYPLQDGFGWTNGVTLKMLDLICPKEQPCDNVPATRPTVKSATTQPSTKEAQPTPHHHHHH

SEQ ID NO: 70 - protein, 1032 aa, Artificial Sequence
  Glucose dehydrogenase N-terminally fused to the TreA with flexible linker and HIS-tag in between GDH and TreA
MAGKYLLPTAAAGLLLLAAQPAMADVPLTPSQFAKAKSENFDKKVILSNLNKPHALLWGPDNQIWLTERATGKILRVNPESGSVKTVFQVPEIVNDADGQNGLLGFAFHPRFKNNPYIYISGTFKNPKSTDKELPNQTIIRRYTYKKKTDTLEKPVDLLAGLPSSKDHQGGRLVIGPDQKIYYTIGDQGRNQFAGLFLPNQAQHTPTQQELNGKDYHTYMGKVLRLNLDGSIPKDNPSFNGVVSHIYTLGHRNPQGLAFTPNGKLLQSDHGPNSDDEINLIVKGGNYGWPNVAGYKDDSGYAYANYSAAANKSIKDLAQNGLKVAAGVPVTKESEWTGKNFVPPLKTLYTVQDTYNYNDPTCGEVTYICWPSVAPSSAYVYKGGKKAITGWENTLLVPSLKRGVIFRIKFDPTYSTTYDDAVPMFKSNNRYRDVIASPDGNVLYVLTDTAGNPVQKDDGSPTNTLENPGSLIKFTYKAKGGKGGSGGSSYAHHHHHHEETPVTPQPPDILLGPLFNDVQNAKLFPDQKTFADAVPNSDPLMILADYRMQQNQSGFDLRHFVNVNFTLPKEGEKYVPPEGQSLREHIDGLWPVLTRSTENTEKWDSLLPLPEPYVVPGGRFREVYYWDSYFTMLGLAESGHWDKVADMVANFAHEIDTYGHIPNGNRSYYLSRSQPPFFALMVELLAQHEGDAALKQYLPQMQKEYAYWMDGVENLQAGQQEKRVVKLQDGTLLNRYWDDRDTPRPESWVEDIATAKSNPNRPATEIYRDLRSAAASGWDFSSRWMDNPQQLNTLRTTSIVPVDLNSLMFKMEKILARASKAAGDNAMANQYETLANARQKGIEKYLWNDQQGWYADYDLKSHKVRNQLTAAALFPLYVNAAAKDRANKMATATKTHLLQPGGLNTTSVKSGQQWDAPNGWAPLQWVATEGLQNYGQKEVAMDISWHFLTNVQHTYDREKKLVEKYDVSTTGTGGGGGEYPLQDGFGWTNGVTLKMLDLICPKEQPCDNVPATRPTVKSATTQPSTKEAQPTP

SEQ ID NO: 71 - protein, 606 aa, Artificial Sequence
  Glucose dehydrogenase N-terminally, and leucine zipper peptide EI C-terminally fused to the N-terminal fragment of TreAN, which with flexible linker and HIS-tag in between GDH and TreAN
MAGKYLLPTAAAGLLLLAAQPAMADVPLTPSQFAKAKSENFDKKVILSNLNKPHALLWGPDNQIWLTERATGKILRVNPESGSVKTVFQVPEIVNDADGQNGLLGFAFHPRFKNNPYIYISGTFKNPKSTDKELPNQTIIRRYTYKKKTDTLEKPVDLLAGLPSSKDHQGGRLVIGPDQKIYYTIGDQGRNQFAGLFLPNQAQHTPTQQELNGKDYHTYMGKVLRLNLDGSIPKDNPSFNGVVSHIYTLGHRNPQGLAFTPNGKLLQSDHGPNSDDEINLIVKGGNYGWPNVAGYKDDSGYAYANYSAAANKSIKDLAQNGLKVAAGVPVTKESEWTGKNFVPPLKTLYTVQDTYNYNDPTCGEVTYICWPSVAPSSAYVYKGGKKAITGWENTLLVPSLKRGVIFRIKFDPTYSTTYDDAVPMFKSNNRYRDVIASPDGNVLYVLTDTAGNPVQKDDGSPTNTLENPGSLIKFTYKAKGGKGGSGGSSYAHHHHHHEETPVTPQPPDILLGPLFNDVQNAKLFPDQKTFADAVPNSDPLMILADYRMQQNQSGFDLRHFVNVNFTLPKEGEKYVPGSEIAALEKEIAALEKENAALEWEIAALEK

SEQ ID NO: 72 - protein, 606 aa, Artificial Sequence
  Glucose dehydrogenase N-terminally, and leucine zipper peptide KI C-terminally fused to the N-terminal fragment of TreAN, which with flexible linker and HIS-tag in between GDH and TreAN
MAGKYLLPTAAAGLLLLAAQPAMADVPLTPSQFAKAKSENFDKKVILSNLNKPHALLWGPDNQIWLTERATGKILRVNPESGSVKTVFQVPEIVNDADGQNGLLGFAFHPRFKNNPYIYISGTFKNPKSTDKELPNQTIIRRYTYKKKTDTLEKPVDLLAGLPSSKDHQGGRLVIGPDQKIYYTIGDQGRNQFAGLFLPNQAQHTPTQQELNGKDYHTYMGKVLRLNLDGSIPKDNPSFNGVVSHIYTLGHRNPQGLAFTPNGKLLQSDHGPNSDDEINLIVKGGNYGWPNVAGYKDDSGYAYANYSAAANKSIKDLAQNGLKVAAGVPVTKESEWTGKNFVPPLKTLYTVQDTYNYNDPTCGEVTYICWPSVAPSSAYVYKGGKKAITGWENTLLVPSLKRGVIFRIKFDPTYSTTYDDAVPMFKSNNRYRDVIASPDGNVLYVLTDTAGNPVQKDDGSPTNTLENPGSLIKFTYKAKGGKGGSGGSSYAHHHHHHEETPVTPQPPDILLGPLFNDVQNAKLFPDQKTFADAVPNSDPLMILADYRMQQNQSGFDLRHFVNVNFTLPKEGEKYVPGSKIAALKEKIAALKEKNAALKWKIAALKE

SEQ ID NO: 73 - protein, 633 aa, Artificial Sequence
  Glucose dehydrogenase N-terminally, and the immunoglobulin binding domain Domain B1 of protein G C-terminally fused to the N-terminal fragment of TreAN, which with flexible linker and HIS-tag in between GDH and TreAN
MAGKYLLPTAAAGLLLLAAQPAMADVPLTPSQFAKAKSENFDKKVILSNLNKPHALLWGPDNQIWLTERATGKILRVNPESGSVKTVFQVPEIVNDADGQNGLLGFAFHPRFKNNPYIYISGTFKNPKSTDKELPNQTIIRRYTYKKKTDTLEKPVDLLAGLPSSKDHQGGRLVIGPDQKIYYTIGDQGRNQFAGLFLPNQAQHTPTQQELNGKDYHTYMGKVLRLNLDGSIPKDNPSFNGVVSHIYTLGHRNPQGLAFTPNGKLLQSDHGPNSDDEINLIVKGGNYGWPNVAGYKDDSGYAYANYSAAANKSIKDLAQNGLKVAAGVPVTKESEWTGKNFVPPLKTLYTVQDTYNYNDPTCGEVTYICWPSVAPSSAYVYKGGKKAITGWENTLLVPSLKRGVIFRIKFDPTYSTTYDDAVPMFKSNNRYRDVIASPDGNVLYVLTDTAGNPVQKDDGSPTNTLENPGSLIKFTYKAKGGKGGSGGSSYAHHHHHHEETPVTPQPPDILLGPLFNDVQNAKLFPDQKTFADAVPNSDPLMILADYRMQQNQSGFDLRHFVNVNFTLPKEGEKYVPGSTYKLILNGKTLKGETTTEAVDAATAEKVFKQYANDNGVDGEWTYDAATKTFTVTE

SEQ ID NO: 74 - protein, 616 aa, Artificial Sequence
  lucose dehydrogenase N-terminally, and the immunoglobulin binding domain Domain B1 of protein G C-terminally fused to the N-terminal fragment of TreAN, which with flexible linker and HIS-tag in between GDH and TreAN
MADVPLTPSQFAKAKSENFDKKVILSNLNKPHALLWGPDNQIWLTERATGKILRVNPESGSVKTVFQVPEIVNDADGQNGLLGFAFHPRFKNNPYIYISGTFKNPKSTDKELPNQTIIRRYTYKKKTDTLEKPVDLLAGLPSSKDHQGGRLVIGPDQKIYYTIGDQGRNQFAGLFLPNQAQHTPTQQELNGKDYHTYMGKVLRLNLDGSIPKDNPSFNGVVSHIYTLGHRNPQGLAFTPNGKLLQSDHGPNSDDEINLIVKGGNYGWPNVAGYKDDSGYAYANYSAAANKSIKDLAQNGLKVAAGVPVTKESEWTGKNFVPPLKTLYTVQDTYNYNDPTCGEVTYICWPSVAPSSAYVYKGGKKAITGWENTLLVPSLKRGVIFRIKFDPTYSTTYDDAVPMFKSNNRYRDVIASPDGNVLYVLTDTAGNPVQKDDGSPTNTLENPGSLIKFTYKAKGGKGGSGGSSYAHHHHHHEETPVTPQPPDILLGPLFNDVQNAKLFPDQKTFADAVPNSDPLMILADYRMQQNQSGFDLRHFVNVNFTLPKEGEKYVPGSTADNKFNKEQQNAFYEILHLPNLNEEQRNGFIQSLKDDPSQSANLLAEAKKLNDAQAPKA

SEQ ID NO: 75 - protein, 643 aa, Artificial Sequence
  Glucose dehydrogenase N-terminally, and the immunoglobulin binding domain B1 of protein G C-terminally fused to the N-terminal fragment of TreAN, which with flexible linker and HIS-tag in between GDH and TreAN
MAGKYLLPTAAAGLLLLAAQPAMADVPLTPSQFAKAKSENFDKKVILSNLNKPHALLWGPDNQIWLTERATGKILRVNPESGSVKTVFQVPEIVNDADGQNGLLGFAFHPRFKNNPYIYISGTFKNPKSTDKELPNQTIIRRYTYKKKTDTLEKPVDLLAGLPSSKDHQGGRLVIGPDQKIYYTIGDQGRNQFAGLFLPNQAQHTPTQQELNGKDYHTYMGKVLRLNLDGSIPKDNPSFNGVVSHIYTLGHRNPQGLAFTPNGKLLQSDHGPNSDDEINLIVKGGNYGWPNVAGYKDDSGYAYANYSAAANKSIKDLAQNGLKVAAGVPVTKESEWTGKNFVPPLKTLYTVQDTYNYNDPTCGEVTYICWPSVAPSSAYVYKGGKKAITGWENTLLVPSLKRGVIFRIKFDPTYSTTYDDAVPMFKSNNRYRDVIASPDGNVLYVLTDTAGNPVQKDDGSPTNTLENPGSLIKFTYKAKGGKGGSGGSSYAHHHHHHEETPVTPQPPDILLGPLFNDVQNAKLFPDQKTFADAVPNSDPLMILADYRMQQNQSGFDLRHFVNVNFTLPKEGEKYVPGSAMEEVTIKANLIFANGSTQTAEFKGTFEKATSEAYAYADTLKKDNGEWTVDVADKGYTLNIKFAG

SEQ ID NO: 76 - protein, 472 aa, Artificial Sequence
  N-terminally HIS-tagged, C-terminally HA-tagged fusion of the N-terminal and C-terminal fragments of TreA in alternative frame folded format
MAHHHHHHNFTLPKEGEKYVPPEGQSLREHIDGSYFTMLGLAESGHWDKVADMVANFAHEIDTYGHIPNGNRSYYLSRSQPPFFALMVELLAQHEGDAALKQYLPQMQKEYAYWMDGVRPESWVEDIATAKSNPNRPATEIYRDLRSAAASGWDFSSRWMDNPQQLNTLRTTSIVPVDLNSLMFKMEKILARASKAAGDNAMANQYETLANARQKGIEKYLWNDQQGWYADYDLKSHKVRNQLTAAALFPLYVNAAAKDRANKMATATKTHLLQPGGLNTTSVKSGQQWDAPNGWAPLQWVATEGLQNYGQKEVAMDISWHFLTNVQHTYDREKKLVEKYDVSTTGTGGGGGEYPLQDGFGWTNGVTLKMLDLICPKEQPEFEETPVTPQPPDILLGPLFNDVQNAKLFPDQKTFADAVPNSDPLMILADYRMQQNQSGFDLRHFVNVNFTLPKEGEKYVPGSYPYDVPDYA

SEQ ID NO: 77 - protein, 542 aa, Artificial Sequence
  N-terminally HA-tagged, C-terminally HIS-tagged fusion of the N-terminal and C-terminal fragments of TreA in alternative frame folded format
MAYPYDVPDYAVDNFTLPKEGEKYVPPEGQSLREHIDGLWPVLTRSTENTEKWDSLLPLPEPYVVPGGRFREVYYWDSYFTMLGLAESGHWDKVADMVANFAHEIDTYGHIPNGNRSYYLSRSQPPFFALMVELLAQHEGDAALKQYLPQMQKEYAYWMDGVENLQAGQQEKRVVKLQDGTLLNRYWDDRDTPRPESWVEDIATAKSNPNRPATEIYRDLRSAAASGWDFSSRWMDNPQQLNTLRTTSIVPVDLNSLMFKMEKILARASKAAGDNAMANQYETLANARQKGIEKYLWNDQQGWYADYDLKSHKVRNQLTAAALFPLYVNAAAKDRANKMATATKTHLLQPGGLNTTSVKSGQQWDAPNGWAPLQWVATEGLQNYGQKEVAMDISWHFLTNVQHTYDREKKLVEKYDVSTTGTGGGGGEYPLQDGFGWTNGVTLKMLDLICPKEQPEFEETPVTPQPPDILLGPLFNDVQNAKLFPDQKTFADAVPNSDPLMILADYRMQQNQSGFDLRHFVNVNFTLPKEGEKYVPHHHHHH

SEQ ID NO: 78 - protein, 561 aa, Artificial Sequence
  N-terminal and C-terminal fragments of TreA in alternative frame folded format with N-terminal and C-terminal fusion with S. aureus binding peptide aptamer and a HIS-tag between both fragments
MVPHNPGLISLQGVDNFTLPKEGEKYVPPEGQSLREHIDGLWPVLTRSTENTEKWDSLLPLPEPYVVPGGRFREVYYWDSYFTMLGLAESGHWDKVADMVANFAHEIDTYGHIPNGNRSYYLSRSQPPFFALMVELLAQHEGDAALKQYLPQMQKEYAYWMDGVENLQAGQQEKRVVKLQDGTLLNRYWDDRDTPRPESWVEDIATAKSNPNRPATEIYRDLRSAAASGWDFSSRWMDNPQQLNTLRTTSIVPVDLNSLMFKMEKILARASKAAGDNAMANQYETLANARQKGIEKYLWNDQQGWYADYDLKSHKVRNQLTAAALFPLYVNAAAKDRANKMATATKTHLLQPGGLNTTSVKSGQQWDAPNGWAPLQWVATEGLQNYGQKEVAMDISWHFLTNVQHTYDREKKLVEKYDVSTTGTGGGGGEYPLQDGFGWTNGVTLKMLDLICPHHHHHHEFEETPVTPEETPVTPQPPDILLGPLFNDVQNAKLFPDQKTFADAVPNSDPLMILADYRMQQNQSGFDLRHFVNVNFTLPKEGEKYVPGSVPHNPGLISLQG

SEQ ID NO: 79 - protein, 712 aa, Artificial Sequence
  Signal Peptide of Aspergillus oryzae fused to glucose oxidase of Aspergillus niger with linker containing HIS-tag to fused to N-terminal fragment of TreA fused to the HA tag
MMVAWWSLFLYGLQVAAPALASNGIEASLLTDPRDVSGRTVDYIIAGGGLTGLTTAARLTENPNISVLVIESGSYESDRGPIIEDLNAYGDIFGSSVDHAYETVELATNNQTALIRSGNGLGGSTLVNGGTWTRPHKAQVDSWETVFGNEGWNWDNVAAYSLQAERARAPNAKQIAAGHYFNASCHGVNGTVHAGPRDTGDDYSPIVKALMSAVEDRGVPTKKDFGCGDPHGVSMFPNTLHEDQVRSDAAREWLLPNYQRPNLQVLTGQYVGKVLLSQNGTTPRAVGVEFGTHKGNTHNVYAKHEVLLAAGSAVSPTILEYSGIGMKSILEPLGIDTVVDLPVGLNLQDQTTATVRSRITSAGAGQGQAAWFATFNETFGDYSEKAHELLNTKLEQWAEEAVARGGFHNTTALLIQYENYRDWIVNHNVAYSELFLDTAGVASFDVWDLLPFTRGYVHILDKDPYLHHFAYDPQYFLNELDLLGQAAATQLARNISNSGAMQTYFAGETIPGDNLAYDADLSAWTEYIPYHFRPNYHGVGTCSMMPKEMGGVVDNAARVYGVQGLRVIDGSIPPTQMSSHVMTVFYAMALKISDAILEDYASMQKGKGGSGGSSYAHHHHHHEETPVTPQPPDILLGPLFNDVQNAKLFPDQKTFADAVPNSDPLMILADYRMQQNQSGFDLRHFVNVNFTLPKEGEKYVPGSYPYDVPDYA